European Patent Specification EP 3 523 333 B1, published December 13, 2023. Title: ANTI-CEACAM6 ANTIBODIES AND METHODS OF USE. Applicant: Agency for Science, Technology and Research. The sequence listing filed with the application follows.

SEQUENCE LISTING (8 sequences)

SEQ ID NO: 1 - protein, 117 aa, Artificial Sequence
  Isolated antibody fragment
SGPELVKPGASVKMSCKASGNTFTSYVMHWVKQKPGQGLEWIGYINPYNDGTKYNEKFKGKATLTSDKSSSTAYMELSSLTSEDSAVYYCARSTARATPYFYAMDYWGQGTSVTVSS

SEQ ID NO: 2 - protein, 115 aa, Artificial Sequence
  Isolated antibody fragment
DILMTQSPSSLAVTAGEKVTMRCKSSQSLLWSVNQNSYLSWYQLKQGQPPKLLLYGASIRESWVPDRFTGSGSGTDFTLTISNVHVEDLAVYYCQHNHGSFLPYTFGGGTKLEIK

SEQ ID NO: 3 - protein, 10 aa, Artificial Sequence
  Isolated antibody fragment
GNTFTSYVMH

SEQ ID NO: 4 - protein, 17 aa, Artificial Sequence
  Isolated antibody fragment
YINPYNDGTKYNEKFKG

SEQ ID NO: 5 - protein, 14 aa, Artificial Sequence
  Isolated antibody fragment
STARATPYFYAMDY

SEQ ID NO: 6 - protein, 16 aa, Artificial Sequence
  Isolated antibody fragment
SSQSLLWSVNQNSYLS

SEQ ID NO: 7 - protein, 7 aa, Artificial Sequence
  Isolated antibody fragment
GASIRES

SEQ ID NO: 8 - protein, 11 aa, Artificial Sequence
  Isolated antibody fragment
QHNHGSFLPYT